European Patent Application EP 4 116 324 A1, published January 11, 2023. Title: Immunoassay Method and Immunoassay Device for Adenovirus. Applicant: Denka Company Limited. The sequence listing filed with the application follows.

SEQUENCE LISTING (12 sequences)

SEQ ID NO: 1 - protein, 6 aa, Adenovirus
NNYYWN

SEQ ID NO: 2 - protein, 16 aa, Adenovirus
YIKYDGSNNNNPSLKN

SEQ ID NO: 3 - protein, 11 aa, Adenovirus
RASYYWDYFDV

SEQ ID NO: 4 - protein, 11 aa, Adenovirus
KANEDIYNGLA

SEQ ID NO: 5 - protein, 7 aa, Adenovirus
GATSLEA

SEQ ID NO: 6 - protein, 9 aa, Adenovirus
QQYWSTPLT

SEQ ID NO: 7 - protein, 5 aa, Adenovirus
NYWIH

SEQ ID NO: 8 - protein, 17 aa, Adenovirus
EIDPTNGRSNYNEKFKT

SEQ ID NO: 9 - protein, 14 aa, Adenovirus
RSYYGSTYDYGLDY

SEQ ID NO: 10 - protein, 16 aa, Adenovirus
RSSKSLLHLNGNTYLY

SEQ ID NO: 11 - protein, 7 aa, Adenovirus
RMSNLAS

SEQ ID NO: 12 - protein, 9 aa, Adenovirus
VQHLEYPYT